European Patent Specification EP 3 763 811 B1, published March 5, 2025. Title: REVERSE TRANSCRIPTASE AND USES THEREOF. Applicant: IRIGEN, S.L.U. The sequence listing filed with the application follows.

SEQUENCE LISTING (1 sequence)

SEQ ID NO: 1 - protein, 683 aa, Artificial sequence
  Artificial sequence
MGSSHHHHHHSSGLEVLFQGPGSTWLSDFPQAWAETGGMGLAVRQAPLIIPLKATSTPVSIKQYPMSQEARLGIKPHIQRLLDQGILVPCQSPWNTPLLPVKKPGTNDYRPVQDLREVNKRVEDIHPTVPNPYNLLSGLPPSHQWYTVLDLKDCFFCLRLHPTSQPLFAFEWRDPEMGISGQLTWTRLPQGFKNSPTLFDEALHRDLADFRIQHPDLILLQYVCDLLLAATSELDCQQGTRALLQTLGNLGYRASAKKAQICQKQVKYLGYLLKEGQRWLTEARKETVMGQPTPKTPRQLREFLGTAGFCRLWIPGFAEMAAPLYPLTKTGTLFNWGPDQQKAYQEIKQALLTAPALGLPDLTKPFELFVDEKQGYAKGVLTQKLGPWRRPVAYLSKKLDPVAAGWPPCLRMVAAIAVLTKDAGKLTMGQPLVILAPHAVEALVKQPPDRWLSNARMTHYQALLLDTDRVQFGPVVALNPATLLPLPEEGLQHNCLDILAEAHGTRPDLTDQPLPDADHTWYTDGSSLLQEGQRKAGAAVTTETEVIWAKALPAGTSAQRAELIALTQALKMAEGKKLNVYTDSRYAFATAHIHGEIYRRRGLLTSEGKEIKNKDEILALLKALFLPKRLSIIHCPGHQKGHSAEARGNRMADQAARKAAITETPDTSTLLIENSSPNSRLIN